European Patent Application EP 4 438 624 A1, published October 2, 2024. Title: Antibodies that bind Nectin-4 and gamma-delta T cell receptors. Applicant: LAVA Therapeutics N.V. The sequence listing filed with the application follows.

SEQUENCE LISTING (76 sequences)

SEQ ID NO: 1 - protein, 118 aa, synthetic construct
EVQLVESGGGLVQAGGSLRLSCAASGSISSINLMGWFRQAPAKQRELVTSISPGGSVRYADSVKGRFTISRDVAKNTVDLQMNSLKPEDTAVYYCAAESERTYYFDSWGQGTQVTVSS

SEQ ID NO: 2 - protein, 5 aa, synthetic construct
INLMG

SEQ ID NO: 3 - protein, 16 aa, synthetic construct
SISPGGSVRYADSVKG

SEQ ID NO: 4 - protein, 10 aa, synthetic construct
ESERTYYFDS

SEQ ID NO: 5 - protein, 30 aa, synthetic construct
EVQLVESGGGLVQAGGSLRLSCAASGSISS

SEQ ID NO: 6 - protein, 14 aa, synthetic construct
WFRQAPAKQRELVT

SEQ ID NO: 7 - protein, 32 aa, synthetic construct
RFTISRDVAKNTVDLQMNSLKPEDTAVYYCAA

SEQ ID NO: 8 - protein, 11 aa, synthetic construct
WGQGTQVTVSS

SEQ ID NO: 9 - protein, 119 aa, synthetic construct
EVQLVESGGGLVQAGGSLRLSCAASGSISSINLMGWHRQAPGKQRELVATITRGGSTNYADSVKGRFTISRDNGKNTVYLQMNSLKPEDTAAYYCVDVEPSGMGWRDYWGQGTQVTVSS

SEQ ID NO: 10 - protein, 5 aa, synthetic construct
INLMG

SEQ ID NO: 11 - protein, 16 aa, synthetic construct
TITRGGSTNYADSVKG

SEQ ID NO: 12 - protein, 11 aa, synthetic construct
VEPSGMGWRDY

SEQ ID NO: 13 - protein, 30 aa, synthetic construct; identical to SEQ ID NO: 5

SEQ ID NO: 14 - protein, 14 aa, synthetic construct
WHRQAPGKQRELVA

SEQ ID NO: 15 - protein, 32 aa, synthetic construct
RFTISRDNGKNTVYLQMNSLKPEDTAAYYCVD

SEQ ID NO: 16 - protein, 11 aa, synthetic construct
WGQGTQVTVSS

SEQ ID NO: 17 - protein, 118 aa, synthetic construct
EVQLVESGGGLVQAGGSLRLSCAASRSTFSLNIMGWYRQAPGKQREYVATITTGGSTNYADSVRGRFTISRDNAEDTVYLQMNSLKPEDTAVYYCTAELVRRGPTTYWGRGTQVTVSS

SEQ ID NO: 18 - protein, 5 aa, synthetic construct
LNIMG

SEQ ID NO: 19 - protein, 16 aa, synthetic construct
TITTGGSTNYADSVRG

SEQ ID NO: 20 - protein, 10 aa, synthetic construct
ELVRRGPTTY

SEQ ID NO: 21 - protein, 30 aa, synthetic construct
EVQLVESGGGLVQAGGSLRLSCAASRSTFS

SEQ ID NO: 22 - protein, 14 aa, synthetic construct
WYRQAPGKQREYVA

SEQ ID NO: 23 - protein, 32 aa, synthetic construct
RFTISRDNAEDTVYLQMNSLKPEDTAVYYCTA

SEQ ID NO: 24 - protein, 11 aa, synthetic construct
WGRGTQVTVSS

SEQ ID NO: 25 - protein, 118 aa, synthetic construct
EVQLVESGGGLVQAGGSLRLSCAASRSTFSLNIMGWYRQAPGKQREYVATITSGGSTNYADSVRGRFTISRDNAENTVYLQMDSLKPEDTAVYYCTAELVRRGPTTYWGRGTQVTVSS

SEQ ID NO: 26 - protein, 5 aa, synthetic construct
LNIMG

SEQ ID NO: 27 - protein, 16 aa, synthetic construct
TITSGGSTNYADSVRG

SEQ ID NO: 28 - protein, 10 aa, synthetic construct
ELVRRGPTTY

SEQ ID NO: 29 - protein, 30 aa, synthetic construct; identical to SEQ ID NO: 21

SEQ ID NO: 30 - protein, 14 aa, synthetic construct
WYRQAPGKQREYVA

SEQ ID NO: 31 - protein, 32 aa, synthetic construct
RFTISRDNAENTVYLQMDSLKPEDTAVYYCTA

SEQ ID NO: 32 - protein, 11 aa, synthetic construct
WGRGTQVTVSS

SEQ ID NO: 33 - protein, 130 aa, synthetic construct
  VARIANT 35: note = X is S or G
  VARIANT 105: note = X can be any amino acid
  VARIANT 109: note = X is not R
EVQLLESGGGSVQPGGSLRLSCAASGRPFSNYAMXWFRQAPGKEREFVSAISWSGGSTSYADSVKGRFTISRDNSKNTLYLQMNSLRAEDTAVYYCAAQFSGADXGFGXLGIRGYEYDYWGQGTQVTVSS

SEQ ID NO: 34 - protein, 5 aa, synthetic construct
  VARIANT 5: note = X is S or G
NYAMX

SEQ ID NO: 35 - protein, 17 aa, synthetic construct
AISWSGGSTSYADSVKG

SEQ ID NO: 36 - protein, 21 aa, synthetic construct
  VARIANT 7: note = X can be any amino acid
  VARIANT 11: note = X is not R
QFSGADXGFGXLGIRGYEYDY

SEQ ID NO: 37 - protein, 130 aa, synthetic construct
EVQLLESGGGSVQPGGSLRLSCAASGRPFSNYAMSWFRQAPGKEREFVSAISWSGGSTSYADSVKGRFTISRDNSKNTLYLQMNSLRAEDTAVYYCAAQFSGADFGFGALGIRGYEYDYWGQGTQVTVSS

SEQ ID NO: 38 - protein, 126 aa, synthetic construct
EVQLVESGGGLVQAGGSLRLSCAASGRPFSNYGMGWFRQAPGKKREFVAGISWSGGSTDYADSVKGRFTISRDNAKNTVYLQMNSLKPEDTAVYYCAAVFSGAETAYYPSDDYDYWGQGTQVTVSS

SEQ ID NO: 39 - protein, 5 aa, synthetic construct
NYGMG

SEQ ID NO: 40 - protein, 17 aa, synthetic construct
GISWSGGSTDYADSVKG

SEQ ID NO: 41 - protein, 17 aa, synthetic construct
VFSGAETAYYPSDDYDY

SEQ ID NO: 42 - protein, 217 aa, synthetic construct
  VARIANT 217: note = X is a K that may or may not be present
APEFEGGPSVFLFPPKPKDTLMISRTPEVTCVVVDVSHEDPEVKFNWYVDGVEVHNAKTKPREEQYNSTYRVVSVLTVLHQDWLNGKEYKCKVSNKALPAPIEKTISKAKGQPREPQVYTLPPSRDELTKNQVSLSCAVKGFYPSDIAVEWESNGQPENNYKTTPPVLDSDGSFFLVSKLTVDKSRWQQGNVFSCSVMHEALHNHYTQKSLSLSPGX

SEQ ID NO: 43 - protein, 217 aa, synthetic construct
  VARIANT 217: note = X is a K that may or may not be present
APEFEGGPSVFLFPPKPKDTLMISRTPEVTCVVVDVSHEDPEVKFNWYVDGVEVHNAKTKPREEQYNSTYRVVSVLTVLHQDWLNGKEYKCKVSNKALPAPIEKTISKAKGQPREPQVYTLPPSRDELTKNQVSLWCLVKGFYPSDIAVEWESNGQPENNYKTTPPVLDSDGSFFLYSKLTVDKSRWQQGNVFSCSVMHEALHNHYTQKSLSLSPGX

SEQ ID NO: 44 - protein, 510 aa, Homo sapiens
MPLSLGAEMWGPEAWLLLLLLLASFTGRCPAGELETSDVVTVVLGQDAKLPCFYRGDSGEQVGQVAWARVDAGEGAQELALLHSKYGLHVSPAYEGRVEQPPPPRNPLDGSVLLRNAVQADEGEYECRVSTFPAGSFQARLRLRVLVPPLPSLNPGPALEEGQGLTLAASCTAEGSPAPSVTWDTEVKGTTSSRSFKHSRSAAVTSEFHLVPSRSMNGQPLTCVVSHPGLLQDQRITHILHVSFLAEASVRGLEDQNLWHIGREGAMLKCLSEGQPPPSYNWTRLDGPLPSGVRVDGDTLGFPPLTTEHSGIYVCHVSNEFSSRDSQVTVDVLDPQEDSGKQVDLVSASVVVVGVIAALLFCLLVVVVVLMSRYHRRKAQQMTQKYEEELTLTRENSIRRLHSHHTDPRSQPEESVGLRAEGHPDSLKDNSSCSVMSEEPEGRSYSTLTTVREIETQTELLSPGSGRAEEEEDQDEGIKQAMNHFVQENGTLRAKPTGNGIYINGRGHLV

SEQ ID NO: 45 - protein, 267 aa, Homo sapiens
MQRISSLIHLSLFWAGVMSAIELVPEHQTVPVSIGVPATLRCSMKGEAIGNYYINWYRKTQGNTMTFIYREKDIYGPGFKDNFQGDIDIAKNLAVLKILAPSERDEGSYYCACDTLGMGGEYTDKLIFGKGTRVTVEPRSQPHTKPSVFVMKNGTNVACLVKEFYPKDIRINLVSSKKITEFDPAIVISPSGKYNAVKLGKYEDSNSVTCSVQHDNKTVHSTDFEVKTDSTDHVKPKETENTKQPSKSCHKPKAIVHTEKVNMMSLT

SEQ ID NO: 46 - protein, 14 aa, synthetic construct
AAASDKTHTCPPCP

SEQ ID NO: 47 - protein, 130 aa, synthetic construct
EVQLVESGGGLVQAGGSLRLSCAASGRPFSNYAMGWFRQAPGKEREFVAAISWSGGSTSYADSVKGRFTISRDNAKNTVYLQMNSPKPEDTAIYYCAAQFSGADYGFGRLGIRGYEYDYWGQGTQVTVSS

SEQ ID NO: 48 - protein, 350 aa, synthetic construct
  VARIANT 350: note = X is a K that may or may not be present
EVQLVESGGGLVQAGGSLRLSCAASGSISSINLMGWHRQAPGKQRELVATITRGGSTNYADSVKGRFTISRDNGKNTVYLQMNSLKPEDTAAYYCVDVEPSGMGWRDYWGQGTQVTVSSAAASDKTHTCPPCPAPEFEGGPSVFLFPPKPKDTLMISRTPEVTCVVVDVSHEDPEVKFNWYVDGVEVHNAKTKPREEQYNSTYRVVSVLTVLHQDWLNGKEYKCKVSNKALPAPIEKTISKAKGQPREPQVYTLPPSRDELTKNQVSLSCAVKGFYPSDIAVEWESNGQPENNYKTTPPVLDSDGSFFLVSKLTVDKSRWQQGNVFSCSVMHEALHNHYTQKSLSLSPGX

SEQ ID NO: 49 - protein, 349 aa, synthetic construct
  VARIANT 349: note = X is a K that may or may not be present
EVQLVESGGGLVQAGGSLRLSCAASGSISSINLMGWFRQAPAKQRELVTSISPGGSVRYADSVKGRFTISRDVAKNTVDLQMNSLKPEDTAVYYCAAESERTYYFDSWGQGTQVTVSSAAASDKTHTCPPCPAPEFEGGPSVFLFPPKPKDTLMISRTPEVTCVVVDVSHEDPEVKFNWYVDGVEVHNAKTKPREEQYNSTYRVVSVLTVLHQDWLNGKEYKCKVSNKALPAPIEKTISKAKGQPREPQVYTLPPSRDELTKNQVSLSCAVKGFYPSDIAVEWESNGQPENNYKTTPPVLDSDGSFFLVSKLTVDKSRWQQGNVFSCSVMHEALHNHYTQKSLSLSPGX

SEQ ID NO: 50 - protein, 349 aa, synthetic construct
  VARIANT 349: note = X is a K that may or may not be present
EVQLVESGGGLVQAGGSLRLSCAASRSTFSLNIMGWYRQAPGKQREYVATITTGGSTNYADSVRGRFTISRDNAEDTVYLQMNSLKPEDTAVYYCTAELVRRGPTTYWGRGTQVTVSSAAASDKTHTCPPCPAPEFEGGPSVFLFPPKPKDTLMISRTPEVTCVVVDVSHEDPEVKFNWYVDGVEVHNAKTKPREEQYNSTYRVVSVLTVLHQDWLNGKEYKCKVSNKALPAPIEKTISKAKGQPREPQVYTLPPSRDELTKNQVSLSCAVKGFYPSDIAVEWESNGQPENNYKTTPPVLDSDGSFFLVSKLTVDKSRWQQGNVFSCSVMHEALHNHYTQKSLSLSPGX

SEQ ID NO: 51 - protein, 349 aa, synthetic construct
  VARIANT 349: note = X is a K that may or may not be present
EVQLVESGGGLVQAGGSLRLSCAASRSTFSLNIMGWYRQAPGKQREYVATITSGGSTNYADSVRGRFTISRDNAENTVYLQMDSLKPEDTAVYYCTAELVRRGPTTYWGRGTQVTVSSAAASDKTHTCPPCPAPEFEGGPSVFLFPPKPKDTLMISRTPEVTCVVVDVSHEDPEVKFNWYVDGVEVHNAKTKPREEQYNSTYRVVSVLTVLHQDWLNGKEYKCKVSNKALPAPIEKTISKAKGQPREPQVYTLPPSRDELTKNQVSLSCAVKGFYPSDIAVEWESNGQPENNYKTTPPVLDSDGSFFLVSKLTVDKSRWQQGNVFSCSVMHEALHNHYTQKSLSLSPGX

SEQ ID NO: 52 - protein, 361 aa, synthetic construct
  VARIANT 361: note = X is a K that may or may not be present
EVQLLESGGGSVQPGGSLRLSCAASGRPFSNYAMSWFRQAPGKEREFVSAISWSGGSTSYADSVKGRFTISRDNSKNTLYLQMNSLRAEDTAVYYCAAQFSGADFGFGALGIRGYEYDYWGQGTQVTVSSAAASDKTHTCPPCPAPEFEGGPSVFLFPPKPKDTLMISRTPEVTCVVVDVSHEDPEVKFNWYVDGVEVHNAKTKPREEQYNSTYRVVSVLTVLHQDWLNGKEYKCKVSNKALPAPIEKTISKAKGQPREPQVYTLPPSRDELTKNQVSLWCLVKGFYPSDIAVEWESNGQPENNYKTTPPVLDSDGSFFLYSKLTVDKSRWQQGNVFSCSVMHEALHNHYTQKSLSLSPGX

SEQ ID NO: 53 - protein, 119 aa, synthetic construct
EVQLVESGGGLVQPGGSLRLSCAASGSISSINLMGWHRQAPGKQRELVATITRGGSTNYADSVKGRFTISRDNGKNTVYLQMNSLRAEDTAAYYCVDVEPSGMGWRDYWGQGTQVTVSS

SEQ ID NO: 54 - protein, 119 aa, synthetic construct
EVQLVESGGGLVQPGGSLRLSCAASGSISSINLMGWHRQAPGKQRELVATITRGGSTNYADSVKGRFTISRDNGKNTLYLQMNSLRAEDTAAYYCVDVEPSGMGWRDYWGQGTQVTVSS

SEQ ID NO: 55 - protein, 119 aa, synthetic construct
EVQLVESGGGLVQPGGSLRLSCAASGSISSINLMGWHRQAPGKGLEWVATITRGGSTNYADSVKGRFTISRDNSKNTLYLQMNSLRAEDTAAYYCVDVEPSGMGWRDYWGQGTLVTVSS

SEQ ID NO: 56 - protein, 118 aa, synthetic construct
EVQLVESGGGLVQPGGSLRLSCAASGSISSINLMGWFRQAPAKQRELVTSISPGGSVRYADSVKGRFTISRDVAKNTVDLQMNSLRAEDTAVYYCAAESERTYYFDSWGQGTQVTVSS

SEQ ID NO: 57 - protein, 118 aa, synthetic construct
EVQLVESGGGLVQPGGSLRLSCAASGSISSINLMGWFRQAPAKQRELVTSISPGGSVRYADSVKGRFTISRDVSKNTVYLQMNSLRAEDTAVYYCAAESERTYYFDSWGQGTQVTVSS

SEQ ID NO: 58 - protein, 118 aa, synthetic construct
EVQLVESGGGLVQPGGSLRLSCAASGSISSINLMGWFRQAPAKGLEWVTSISPGGSVRYADSVKGRFTISRDNSKNTLYLQMNSLRAEDTAVYYCAAESERTYYFDSWGQGTQVTVSS

SEQ ID NO: 59 - protein, 118 aa, synthetic construct
EVQLVESGGGLVQPGGSLRLSCAASRSTFSLNIMGWYRQAPGKQREYVATITTGGSTNYADSVRGRFTISRDNAEDTVYLQMNSLRAEDTAVYYCTAELVRRGPTTYWGRGTQVTVSS

SEQ ID NO: 60 - protein, 118 aa, synthetic construct
EVQLVESGGGLVQPGGSLRLSCAASRSTFSLNIMGWYRQAPGKQREYVATITTGGSTNYADSVRGRFTISRDNSEDTVYLQMNSLRAEDTAVYYCTAELVRRGPTTYWGRGTQVTVSS

SEQ ID NO: 61 - protein, 118 aa, synthetic construct
EVQLVESGGGLVQPGGSLRLSCAASRSTFSLNIMGWYRQAPGKQREYVATITTGGSTNYADSVRGRFTISRDNSKNTLYLQMNSLRAEDTAVYYCTAELVRRGPTTYWGRGTLVTVSS

SEQ ID NO: 62 - protein, 118 aa, synthetic construct
EVQLVESGGGLVQPGGSLRLSCAASRSTFSLNIMGWYRQAPGKQREYVATITSGGSTNYADSVRGRFTISRDNAENTVYLQMDSLRAEDTAVYYCTAELVRRGPTTYWGRGTQVTVSS

SEQ ID NO: 63 - protein, 118 aa, synthetic construct
EVQLVESGGGLVQPGGSLRLSCAASRSTFSLNIMGWYRQAPGKQREYVATITSGGSTNYADSVRGRFTISRDNSENTVYLQMDSLRAEDTAVYYCTAELVRRGPTTYWGRGTQVTVSS

SEQ ID NO: 64 - protein, 118 aa, synthetic construct
EVQLVESGGGLVQPGGSLRLSCAASRSTFSLNIMGWYRQAPGKGLEWVATITSGGSTNYADSVRGRFTISRDNSKNTLYLQMDSLRAEDTAVYYCTAELVRRGPTTYWGRGTLVTVSS

SEQ ID NO: 65 - protein, 124 aa, synthetic construct
EVQLVESGGALVQAGGSLRLSCSVSGLTASRLTMGWFRQAPGKEREFVARVYASGGLTDYADSVKGRFTISRDNAKNTVYLQMNSLEPEDTAVYYCVAGLWADMRTMTSTRGYWGQGTQVTVSS

SEQ ID NO: 66 - protein, 5 aa, synthetic construct
RLTMG

SEQ ID NO: 67 - protein, 17 aa, synthetic construct
RVYASGGLTDYADSVKG

SEQ ID NO: 68 - protein, 15 aa, synthetic construct
GLWADMRTMTSTRGY

SEQ ID NO: 69 - protein, 118 aa, synthetic construct
EVQLVESGGGLVQAGGSLRLSCAASGSIFDINLMGWYRQAPGKLRELVASITRGGSTWYVDSVKGRFIISRDSAKNTVYLQMNSLKPGDTAVYYCAAESIGSYTFDRWGQGTQVTVSS

SEQ ID NO: 70 - protein, 5 aa, synthetic construct
INLMG

SEQ ID NO: 71 - protein, 16 aa, synthetic construct
SITRGGSTWYVDSVKG

SEQ ID NO: 72 - protein, 10 aa, synthetic construct
ESIGSYTFDR

SEQ ID NO: 73 - protein, 117 aa, synthetic construct
EVQLVESGGGLVQAGGFLRLSCAASRSVFRINVMGWYRQAPGKQRELVAGITSGGSRRLADSVKGRFTISRDNAKNTVYLQMNSLKPEDTAVYYCFAEAVVGDEPYWGQGTQVTVSS

SEQ ID NO: 74 - protein, 5 aa, synthetic construct
INVMG

SEQ ID NO: 75 - protein, 16 aa, synthetic construct
GITSGGSRRLADSVKG

SEQ ID NO: 76 - protein, 9 aa, synthetic construct
EAVVGDEPY